European Patent Specification EP 3 150 631 B1, published August 30, 2023. Title: ANTI-GLUCOSAMINIDASE PASSIVE IMMUNIZATION FOR STAPHYLOCOCCUS AUREUS INFECTIONS. Applicant: University of Rochester. The sequence listing filed with the application follows.

SEQUENCE LISTING (36 sequences)

SEQ ID NO: 1 - protein, 148 aa, Mus musculus
  MISC_FEATURE (145)..(145): X at position 145 is any amino acid
EVQLQESGPVLVKPGASVKMSCKASGYTFTDYYMNWVKQSHGKSLEWIGVINPYNGDTTYSQKFKGKATLTVDKSSSTAYMELNSLTSEDSAVYYCARNYDEYFDVWGTGTTVTVSSAKTTPPSVYPLAPGSAAQTNSMVTLGCXVKG

SEQ ID NO: 2 - protein, 155 aa, Mus musculus
  MISC_FEATURE (153)..(153): X at position 153 is any amino acid
EVQLQESGPVLVKPGASVKLSCKASGYTFTDYFMNWVKQSHGKSLEWIGVINPFNGGNRYNQNFKGKATLTVDKSSSTAYMELNSLTSEDSAVYYCARGDYDSPWFDYWGQGTLVTVSAAKTTPPSVYPLAPGSAAQTNSMVTLGCLVKGYSXSQ

SEQ ID NO: 3 - protein, 152 aa, Mus musculus
EVQLQESGGGFVKPGGSLKLSCAASGFTFSTYVMSWVRQTPEKRLEWVATISDGGGHTYYLDNVKGRFTISRDNAKNNLYLHMSHLKSEDTAMYYCARAYYGSSYDAMDYWGQGTSVTVSSAKTTPPSVYPLAPGSAAQTNSMVTLGCLVKG

SEQ ID NO: 4 - protein, 152 aa, Mus musculus
EVQLQESGGGLVQPGGSMKLSCAASGFTFSDAWMDWVRQSPEKGLEWVAEIKDKTNNHATYYAESVKGRFTISRDVSKSRVFLQMNSLRPEDTGIYYCTSGPYFDYWGQGTTLTVSSAKTTPPSVYPLAPGSAAQTNSMVTLGCLVKGYFPE

SEQ ID NO: 5 - protein, 122 aa, Mus musculus
QIQLVQSGPELKKPGETVKISCKASGYTFTTYGMSWVNQAPGKGLKWMGWINTYSGVPTYADDFKGRFVFSLETSASTAYLQINNLKNEDTATYFCAREEYSSGYAAWFPYWGQGTLVTVSA

SEQ ID NO: 6 - protein, 160 aa, Artificial sequence
  Consensus alignment of SEQ ID NOS: 1-5
  MISC_FEATURE (1)..(2): X at position 1 to 2 is any amino acid
  MISC_FEATURE (5)..(6): X at position 5 to 6 is any amino acid
  MISC_FEATURE (9)..(13): X at position 9 to 13 is any amino acid
  MISC_FEATURE (16)..(18): X at position 16 to 18 is any amino acid
  MISC_FEATURE (20)..(20): X at position 20 is any amino acid
  MISC_FEATURE (23)..(23): X at position 23 is any amino acid
  MISC_FEATURE (27)..(27): X at position 27 is any amino acid
  MISC_FEATURE (30)..(33): X at position 30 to 33 is any amino acid
  MISC_FEATURE (35)..(35): X at position 35 is any amino acid
  MISC_FEATURE (38)..(38): X at position 38 is any amino acid
  MISC_FEATURE (40)..(42): X at position 40 to 42 is any amino acid
  MISC_FEATURE (44)..(44): X at position 44 is any amino acid
  MISC_FEATURE (46)..(46): X at position 46 is any amino acid
  MISC_FEATURE (48)..(50): X at position 48 to 50 is any amino acid
  MISC_FEATURE (52)..(61): X at position 52 to 61 is any amino acid
  MISC_FEATURE (63)..(66): X at position 63 to 66 is any amino acid
  MISC_FEATURE (69)..(87): X at position 69 to 87 is any amino acid
  MISC_FEATURE (89)..(90): X at position 89 to 90 is any amino acid
  MISC_FEATURE (93)..(95): X at position 93 to 95 is any amino acid
  MISC_FEATURE (97)..(97): X at position 97 is any amino acid
  MISC_FEATURE (99)..(102): X at position 99 to 102 is any amino acid
  MISC_FEATURE (103)..(112): X at position 103 to 112 is any amino acid
  misc_feature (113)..(113): Xaa can be any naturally occurring amino acid
  MISC_FEATURE (115)..(115): X at position 115 is any amino acid
  misc_feature (116)..(116): Xaa can be any naturally occurring amino acid
  MISC_FEATURE (118)..(119): X at position 118 to 119 is any amino acid
  misc_feature (120)..(120): Xaa can be any naturally occurring amino acid
  MISC_FEATURE (123)..(159): X at position 123 to 159 is any amino acid
  misc_feature (160)..(160): Xaa can be any naturally occurring amino acid
XXQLXXSGXXXXXPGXXXKXSCXASGXTFXXXXMXWVXQXXXKXLXWXXXIXXXXXXXXXXYXXXXKGXXXXXXXXXXXXXXXXXXXLXXEDXXXYXCXXXXYXXXXXXXXXXWGXGTXXTVSXXXXXXXXXXXXXXXXXXXXXXXXXXXXXXXXXXXXX

SEQ ID NO: 7 - protein, 159 aa, Artificial sequence
  Consensus alignment of SEQ ID NOS: 4-5
  MISC_FEATURE (1)..(2): X at position 1 to 2 is any amino acid
  MISC_FEATURE (5)..(6): X at position 5 to 6 is any amino acid
  MISC_FEATURE (9)..(10): X at position 9 to 10 is any amino acid
  MISC_FEATURE (12)..(13): X at position 12 to 13 is any amino acid
  MISC_FEATURE (16)..(20): X at position 16 to 20 is any amino acid
  MISC_FEATURE (23)..(23): X at position 23 is any amino acid
  MISC_FEATURE (27)..(27): X at position 27 is any amino acid
  MISC_FEATURE (30)..(33): X at position 30 to 33 is any amino acid
  MISC_FEATURE (35)..(35): X at position 35 is any amino acid
  MISC_FEATURE (38)..(38): X at position 38 is any amino acid
  MISC_FEATURE (40)..(40): X at position 40 is any amino acid
  MISC_FEATURE (42)..(42): X at position 42 is any amino acid
  MISC_FEATURE (46)..(46): X at position 46 is any amino acid
  MISC_FEATURE (48)..(50): X at position 48 to 50 is any amino acid
  MISC_FEATURE (52)..(54): X at position 52 to 54 is any amino acid
  MISC_FEATURE (56)..(61): X at position 56 to 61 is any amino acid
  MISC_FEATURE (64)..(66): X at position 64 to 66 is any amino acid
  MISC_FEATURE (71)..(72): X at position 71 to 72 is any amino acid
  MISC_FEATURE (74)..(76): X at position 74 to 76 is any amino acid
  MISC_FEATURE (78)..(78): X at position 78 is any amino acid
  MISC_FEATURE (80)..(82): X at position 80 to 82 is any amino acid
  MISC_FEATURE (85)..(85): X at position 85 is any amino acid
  MISC_FEATURE (87)..(87): X at position 87 is any amino acid
  MISC_FEATURE (89)..(90): X at position 89 to 90 is any amino acid
  MISC_FEATURE (94)..(95): X at position 94 to 95 is any amino acid
  MISC_FEATURE (97)..(97): X at position 97 is any amino acid
  MISC_FEATURE (99)..(104): X at position 99 to 104 is any amino acid
  MISC_FEATURE (107)..(110): X at position 107 to 110 is any amino acid
  MISC_FEATURE (112)..(112): X at position 112 is any amino acid
  MISC_FEATURE (119)..(120): X at position 119 to 120 is any amino acid
  MISC_FEATURE (124)..(159): X at position 124 to 159 is any amino acid
XXQLXXSGXXLXXPGXXXKXSCXASGXTFXXXXMXWVXQXPXKGLXWXXXIXXXTXXXXXXYAXXXKGRFXXSXXXSXSXXXLQXNXLXXEDTXXYXCXXXXXXSGXXXXFXYWGQGTXXTVSXXXXXXXXXXXXXXXXXXXXXXXXXXXXXXXXXXXX

SEQ ID NO: 8 - protein, 98 aa, Mus musculus
DIVMTQSPAIMSASPGEKVTMTCSASSSVSYMYWYQQKPGSSPRLLIYDTSNLASGVPVRFSGSGSGTSYSLTISRMEAEDAATYYCQQWSSYPLTFG

SEQ ID NO: 9 - protein, 105 aa, Mus musculus
QMTQTTSSLSASLGDRVTISCSASQGISNYLNWYQQKPDGTVKLLIYYTSSLHSGVPSRFSGGGSGTDYSLSISNLEPEDIATYYCQQYSKLPWTFGGGTKLEIK

SEQ ID NO: 10 - protein, 103 aa, Mus musculus
  MISC_FEATURE (47)..(47): X at position 47 is any amino acid
DIVITQSPAIMSASLGERVTMTCTASSSVSSSYLHWYQQKPGSSPKXWIYSTSNLASGVPARFSGSGSGTSYSLTISSMEAEDAATYYCHQYHRSPWTFGGGT

SEQ ID NO: 11 - protein, 107 aa, Mus musculus
DIVMTQSHKFMSTSVGDRVSITCKASQDVSTAVAWYQQKPGQSPKLLIYWTSTRHTGVPDRFTGSGSGTDFTLTISSVQAKDLALYYCQQHYTTPYTFGGGTKLEIK

SEQ ID NO: 12 - protein, 107 aa, Mus musculus
DIVLTQSPATLSVTPGDSVSLSCRASQSISNNLHWYQQKSHESPRLLIEYASRSISGIPSRFSGGGSGTDFTLSINSVESEDFGLYFCQQSNSWPLTFGAGTKLELK

SEQ ID NO: 13 - protein, 108 aa, Artificial sequence
  Consensus alignment of SEQ ID NOS: 8-12
  MISC_FEATURE (3)..(4): X at position 3 to 4 is any amino acid or a deletion
  MISC_FEATURE (7)..(11): X at position 7 to 11 is any amino acid or a deletion
  MISC_FEATURE (13)..(15): X at position 13 to 15 is any amino acid or a deletion
  MISC_FEATURE (17)..(18): X at position 17 to 18 is any amino acid or a deletion
  MISC_FEATURE (20)..(22): X at position 20 to 22 is any amino acid or a deletion
  MISC_FEATURE (24)..(24): X at position 24 is any amino acid or a deletion
  MISC_FEATURE (27)..(29): X at position 27 to 29 is any amino acid or a deletion
  MISC_FEATURE (31)..(35): X at position 31 to 35 is any amino acid or a deletion
  MISC_FEATURE (41)..(48): X at position 41 to 48 is any amino acid or a deletion
  MISC_FEATURE (50)..(52): X at position 50 to 52 is any amino acid or a deletion
  MISC_FEATURE (54)..(57): X at position 54 to 57 is any amino acid or a deletion
  MISC_FEATURE (59)..(59): X at position 59 is any amino acid or a deletion
  MISC_FEATURE (61)..(61): X at position 61 is any amino acid or a deletion
  MISC_FEATURE (64)..(64): X at position 64 is any amino acid or a deletion
  MISC_FEATURE (66)..(66): X at position 66 is any amino acid or a deletion
  MISC_FEATURE (71)..(73): X at position 71 to 73 is any amino acid or a deletion
  MISC_FEATURE (75)..(75): X at position 75 is any amino acid or a deletion
  MISC_FEATURE (77)..(82): X at position 77 to 82 is any amino acid or a deletion
  MISC_FEATURE (84)..(86): X at position 84 to 86 is any amino acid or a deletion
  MISC_FEATURE (88)..(88): X at position 88 is any amino acid or a deletion
  MISC_FEATURE (90)..(90): X at position 90 is any amino acid or a deletion
  MISC_FEATURE (92)..(95): X at position 92 to 95 is any amino acid or a deletion
  MISC_FEATURE (97)..(97): X at position 97 is any amino acid or a deletion
  MISC_FEATURE (101)..(101): X at position 101 is any amino acid or a deletion
  MISC_FEATURE (104)..(108): X at position 104 to 108 is any amino acid or a deletion
DIXXTQXXXXXSXXXGXXVXXXCXASXXXSXXXXXWYQQKXXXXXXXXIXXXSXXXXGXPXRFXGXGSGTXXXLXIXXXXXXDXXXYXCXQXXXXPXTFGXGTXXXXX

SEQ ID NO: 14 - protein, 107 aa, Artificial Sequence
  Consensus alignment of SEQ ID NOS: 11-12
  MISC_FEATURE (4)..(4): X at position 4 is any amino acid or a deletion
  MISC_FEATURE (8)..(11): X at position 8 to 11 is any amino acid or a deletion
  MISC_FEATURE (13)..(15): X at position 13 to 15 is any amino acid or a deletion
  MISC_FEATURE (18)..(18): X at position 18 is any amino acid or a deletion
  MISC_FEATURE (21)..(22): X at position 21 to 22 is any amino acid or a deletion
  MISC_FEATURE (24)..(24): X at position 24 is any amino acid or a deletion
  MISC_FEATURE (28)..(29): X at position 28 to 29 is any amino acid or a deletion
  MISC_FEATURE (31)..(34): X at position 31 to 34 is any amino acid or a deletion
  MISC_FEATURE (40)..(42): X at position 40 to 42 is any amino acid or a deletion
  MISC_FEATURE (45)..(45): X at position 45 is any amino acid or a deletion
  MISC_FEATURE (49)..(51): X at position 49 to 51 is any amino acid or a deletion
  MISC_FEATURE (53)..(56): X at position 53 to 56 is any amino acid or a deletion
  MISC_FEATURE (58)..(58): X at position 58 is any amino acid or a deletion
  MISC_FEATURE (60)..(60): X at position 60 is any amino acid or a deletion
  MISC_FEATURE (63)..(63): X at position 63 is any amino acid or a deletion
  MISC_FEATURE (65)..(65): X at position 65 is any amino acid or a deletion
  MISC_FEATURE (74)..(74): X at position 74 is any amino acid or a deletion
  MISC_FEATURE (76)..(76): X at position 76 is any amino acid or a deletion
  MISC_FEATURE (79)..(81): X at position 79 to 81 is any amino acid or a deletion
  MISC_FEATURE (83)..(84): X at position 83 to 84 is any amino acid or a deletion
  MISC_FEATURE (87)..(87): X at position 87 is any amino acid or a deletion
  MISC_FEATURE (91)..(94): X at position 91 to 94 is any amino acid or a deletion
  MISC_FEATURE (96)..(96): X at position 96 is any amino acid or a deletion
  MISC_FEATURE (100)..(100): X at position 100 is any amino acid or a deletion
  MISC_FEATURE (106)..(106): X at position 106 is any amino acid or a deletion
DIVXTQSXXXXSXXXGDXVSXXCXASQXXSXXXXWYQQKXXXSPXLLIXXXSXXXXGXPXRFXGXGSGTDFTLXIXSVXXXDXXLYXCQQXXXXPXTFGXGTKLEXK

SEQ ID NO: 15 - protein, 21 aa, Artificial Sequence
  Primer for S. aureus nuc gene
GCGATTGATGGTGATACGGTT

SEQ ID NO: 16 - protein, 21 aa, Artificial Sequence
  Primer for S. aureus nuc gene
AGCCAAGCCTTGACGAACTAA

SEQ ID NO: 17 - protein, 20 aa, Artificial Sequence
  Primer for mouse b-actin gene
AGATGTGAATCAGCAAGCAG

SEQ ID NO: 18 - protein, 20 aa, Artificial Sequence
  Primer for mouse b-actin gene
GCGCAAGTTAGGTTTTGTCA

SEQ ID NO: 19 - protein, 110 aa, Homo sapiens
QVQLVQSGHEVKQPGASVKVSCKASGYSFTTYGMNWVPQAPGQGLEWMGWFNTYTGNPTYAQGFTGRFVFSMDTSASTAYLQISSLKAEDMAMYYCARYWGQGTLVTVSA

SEQ ID NO: 20 - protein, 107 aa, Homo sapiens
EIVLTQSPDFQSVTPKEKVTITCRASQSIGSSLHWYQQKPDQSPKLLIKYASQSFSGVPSRFSGSGSGTDFTLTINSLEAEDAATYYCHQSSSLPLTFGGGTKVEIK

SEQ ID NO: 21 - DNA, 444 bp, Mus musculus
  misc_feature (434)..(434): N at position 434 is unknown
gaggtgcagctgcaggagtctggacctgtgctggtgaagcctggggcttcagtgaagatgtcctgtaaggcttctggatacacattcactgactactatatgaactgggtgaagcagagccatggaaagagccttgagtggattggagttattaatccttacaacggtgatactacctacagccagaagttcaagggcaaggccacattgactgttgacaagtcctccagcacagcctacatggagctcaacagcctgacatctgaggactctgcagtctattactgtgcaagaaattacgacgagtacttcgatgtctggggcacagggaccacggtcaccgtctcctcagccaaaacgacacccccatctgtctatccactggcccctggatctgctgcccaaactaactccatggtgaccctgggatgccnggtcaagggc

SEQ ID NO: 22 - DNA, 294 bp, Mus musculus
gatattgtgatgacccagtctccagcaatcatgtctgcatctccaggggagaaggtcaccatgacctgcagtgccagctcaagtgtaagttacatgtactggtaccagcagaagccaggatcctcccccagactcctgatttatgacacatccaacctggcttctggagtccctgttcgcttcagtggcagtgggtctgggacctcttactctctcacaatcagccgaatggaggctgaggatgctgccacttattactgccagcagtggagtagttacccgctcacgttcggt

SEQ ID NO: 23 - DNA, 467 bp, Mus musculus
  misc_feature (458)..(458): N at position 458 is unknown
gaggtgcagctgcaggagtctggacctgtgctggtgaagcctggggcttcagtgaagctgtcctgtaaggcttctggatacacattcactgactactttatgaactgggtgaagcagagccatggaaagagccttgagtggattggagttattaatcctttcaacggtggtaataggtacaaccagaacttcaagggcaaggccacattgactgttgacaagtcctccagcacagcctacatggagctcaacagcctgacatctgaggactctgcagtctattactgtgcaagaggggactatgactccccctggtttgattactggggccaagggactctggtcactgtctctgcagccaaaacgacacccccatctgtctatccactggcccctggatctgctgcccaaactaactccatggtgaccctgggatgcctggtcaagggctattcccngagccagtg

SEQ ID NO: 24 - DNA, 315 bp, Mus musculus
cagatgacacagactacgtcctccctgtctgcctctctgggagacagagtcaccatcagttgcagtgcaagtcagggcattagcaattatttaaactggtatcagcagaaaccagatggaactgttaaactcctgatctattacacatcaagtttacactcaggagtcccatcaaggttcagtggcggtgggtctgggacagattattctctctccatcagcaacctggaacctgaagatattgccacttactattgtcagcagtatagtaagcttccttggacgttcggtggaggcaccaagctggaaatcaaa

SEQ ID NO: 25 - DNA, 456 bp, Mus musculus
gaggtgcagctgcaggagtctgggggaggcttcgtgaagcctggagggtccctgaaactctcctgtgcagcctctggattcactttcagtacctatgtcatgtcttgggttcgccagactccggaaaagaggctggagtgggtcgcaaccattagtgatggtggtggtcatacttactatctagacaatgtaaagggccgattcaccatctccagagacaatgccaagaacaacctgtacctgcacatgagccatctgaagtctgaggacacagccatgtattactgtgcaagagcttactacggtagtagttacgacgctatggactactggggtcaaggaacctcagtcaccgtctcctcagccaaaacgacacccccatctgtctatccactggcccctggatctgctgcccaaactaactccatggtgaccctgggatgcctggtcaagggc

SEQ ID NO: 26 - DNA, 309 bp, Mus musculus
  misc_feature (141)..(141): N at position 141 is unknown
gatattgtgatcacccagtctccagcaatcatgtctgcatctctaggggaacgggtcaccatgacctgcactgccagctcaagtgtaagttccagttacttacactggtaccagcagaagccaggatcctcccccaaactntggatttatagcacatccaacctggcttctggagtcccagctcgcttcagtggcagtgggtctgggacctcttactctctcacaatcagcagcatggaggctgaagatgctgccacttattactgccaccagtatcatcgttccccatggacgttcggtggaggcacc

SEQ ID NO: 27 - DNA, 456 bp, Mus musculus
gaggtgcagctgcaggagtctggaggaggcttggtgcaacctggaggatccatgaaactctcttgtgctgcctctggattcacttttagtgacgcctggatggactgggtccgccagtctccagagaaggggcttgagtgggttgctgaaattaaagacaaaactaataatcatgcaacatactatgctgagtctgtgaaagggaggttcaccatctcaagagatgtttccaaaagtcgtgtcttcctgcaaatgaacagcttaagacctgaagacactggcatttattactgtacgtctgggccatattttgactactggggccaaggcaccactctcacagtctcctcagccaaaacgacacccccatctgtctatccactggcccctggatctgctgcccaaactaactccatggtgaccctgggatgcctggtcaagggctatttccctgag

SEQ ID NO: 28 - DNA, 321 bp, Mus musculus
gacattgtgatgacccagtctcacaaattcatgtccacatcagtaggagacagggtcagcatcacctgcaaggccagtcaggacgtgagtactgctgtagcctggtatcaacaaaaaccagggcaatctcctaaactactgatttactggacatccacccggcacactggagtccctgatcgcttcacaggcagtggatctgggacagattttactctcaccatcagcagtgtgcaggctaaagacctggcactttattactgtcagcaacattataccactccgtacacgttcggaggggggaccaagctggaaataaaa

SEQ ID NO: 29 - DNA, 366 bp, Mus musculus
cagatccagttggtacagtctggacctgagctgaagaagcctggagagacagtcaagatctcctgcaaggcttctgggtataccttcacaacgtatggaatgagctgggtgaatcaggctccaggaaagggtttaaagtggatgggctggataaacacctactctggagtgccaacatatgctgatgacttcaagggacggtttgtcttctctttggaaacctctgccagcactgcctatttgcagatcaacaacctcaaaaatgaggacacggctacatatttctgtgcaagagaggagtacagctcaggctacgcggcctggtttccttactggggccaagggactctggtcactgtctctgca

SEQ ID NO: 30 - DNA, 321 bp, Mus musculus
gatattgtgctaactcagtctccagccaccctgtctgtgactccaggagatagcgtcagtctttcctgcagggccagccaaagtattagcaacaacctacactggtatcaacaaaaatcacatgagtctccaaggcttctcatcgaatatgcttcccggtccatctctgggatcccctctaggttcagtggcggtggatcagggacagatttcactctcagtatcaacagtgtggagtctgaagattttggattgtatttctgtcaacagagtaacagctggccgctcacgttcggtgctgggaccaagctggagctgaaa

SEQ ID NO: 31 - protein, 159 aa, Artificial Sequence
  Consensus alignment of SEQ ID NOS: 1-4
  MISC_FEATURE (9)..(11): X at position 9 to 11 is any amino acid
  MISC_FEATURE (13)..(13): X at position 13 is any amino acid
  MISC_FEATURE (16)..(16): X at position 16 is any amino acid
  MISC_FEATURE (18)..(18): X at position 18 is any amino acid
  MISC_FEATURE (20)..(20): X at position 20 is any amino acid
  MISC_FEATURE (23)..(23): X at position 23 is any amino acid
  MISC_FEATURE (27)..(27): X at position 27 is any amino acid
  MISC_FEATURE (30)..(33): X at position 30 to 33 is any amino acid
  MISC_FEATURE (35)..(35): X at position 35 is any amino acid
  MISC_FEATURE (38)..(38): X at position 38 is any amino acid
  MISC_FEATURE (40)..(42): X at position 40 to 42 is any amino acid
  MISC_FEATURE (44)..(44): X at position 44 is any amino acid
  MISC_FEATURE (48)..(61): X at position 48 to 61 is any amino acid
  MISC_FEATURE (63)..(66): X at position 63 to 66 is any amino acid
  MISC_FEATURE (69)..(70): X at position 69 to 70 is any amino acid
  MISC_FEATURE (72)..(74): X at position 72 to 74 is any amino acid
  MISC_FEATURE (76)..(87): X at position 76 to 87 is any amino acid
  MISC_FEATURE (89)..(90): X at position 89 to 90 is any amino acid
  MISC_FEATURE (93)..(95): X at position 93 to 95 is any amino acid
  MISC_FEATURE (99)..(102): X at position 99 to 102 is any amino acid
  MISC_FEATURE (104)..(110): X at position 104 to 110 is any amino acid
  MISC_FEATURE (112)..(112): X at position 112 is any amino acid
  MISC_FEATURE (115)..(115): X at position 115 is any amino acid
  MISC_FEATURE (118)..(119): X at position 118 to 119 is any amino acid
  MISC_FEATURE (123)..(123): X at position 123 is any amino acid
  MISC_FEATURE (151)..(151): X at position 151 is any amino acid
  MISC_FEATURE (155)..(159): X at position 155 to 159 is any amino acid
EVQLQESGXXXVXPGXSXKXSCXASGXTFXXXXMXWVXQXXXKXLEWXXXIXXXXXXXXXXYXXXXKGXXTXXXDXXXXXXXXXXXXLXXEDXXXYYCXXXXYXXXXXXXDXWGXGTXXTVSXAKTTPPSVYPLAPGSAAQTNSMVTLGCXVKGXXXXX

SEQ ID NO: 32 - protein, 103 aa, Artificial Sequence
  Consensus alignment of SEQ ID NOS: 8 and 10
  MISC_FEATURE (4)..(4): X at position 4 is any amino acid or a deletion
  MISC_FEATURE (15)..(15): X at position 15 is any amino acid or a deletion
  MISC_FEATURE (18)..(18): X at position 18 is any amino acid or a deletion
  MISC_FEATURE (24)..(24): X at position 24 is any amino acid or a deletion
  MISC_FEATURE (31)..(32): X at position 31 to 32 is any amino acid or a deletion
  MISC_FEATURE (34)..(35): X at position 34 to 35 is any amino acid or a deletion
  MISC_FEATURE (46)..(48): X at position 46 to 48 is any amino acid or a deletion
  MISC_FEATURE (51)..(51): X at position 51 is any amino acid or a deletion
  MISC_FEATURE (61)..(61): X at position 61 is any amino acid or a deletion
  MISC_FEATURE (78)..(78): X at position 78 is any amino acid or a deletion
  MISC_FEATURE (90)..(90): X at position 90 is any amino acid or a deletion
  MISC_FEATURE (92)..(95): X at position 92 to 95 is any amino acid or a deletion
  MISC_FEATURE (97)..(97): X at position 97 is any amino acid or a deletion
  MISC_FEATURE (101)..(103): X at position 101 to 103 is any amino acid or a deletion
DIVXTQSPAIMSASXGEXVTMTCXASSSVSXXYXXWYQQKPGSSPXXXIYXTSNLASGVPXRFSGSGSGTSYSLTISXMEAEDAATYYCXQXXXXPXTFGXXX

SEQ ID NO: 33 - protein, 109 aa, Artificial Sequence
  Consensus alignment of SEQ ID NOS: 8-11
  MISC_FEATURE (3)..(4): X at position 3 to 4 is any amino acid or a deletion
  MISC_FEATURE (7)..(11): X at position 7 to 11 is any amino acid or a deletion
  MISC_FEATURE (13)..(13): X at position 13 is any amino acid or a deletion
  MISC_FEATURE (15)..(15): X at position 15 is any amino acid or a deletion
  MISC_FEATURE (17)..(18): X at position 17 to 18 is any amino acid or a deletion
  MISC_FEATURE (20)..(22): X at position 20 to 22 is any amino acid or a deletion
  MISC_FEATURE (24)..(24): X at position 24 is any amino acid or a deletion
  MISC_FEATURE (27)..(29): X at position 27 to 29 is any amino acid or a deletion
  MISC_FEATURE (31)..(35): X at position 31 to 35 is any amino acid or a deletion
  MISC_FEATURE (42)..(48): X at position 42 to 48 is any amino acid or a deletion
  MISC_FEATURE (51)..(51): X at position 51 is any amino acid or a deletion
  MISC_FEATURE (54)..(57): X at position 54 to 57 is any amino acid or a deletion
  MISC_FEATURE (62)..(62): X at position 62 is any amino acid or a deletion
  MISC_FEATURE (65)..(65): X at position 65 is any amino acid or a deletion
  MISC_FEATURE (67)..(67): X at position 67 is any amino acid or a deletion
  MISC_FEATURE (72)..(74): X at position 72 to 74 is any amino acid or a deletion
  MISC_FEATURE (76)..(76): X at position 76 is any amino acid or a deletion
  MISC_FEATURE (79)..(83): X at position 79 to 83 is any amino acid or a deletion
  MISC_FEATURE (85)..(85): X at position 85 is any amino acid or a deletion
  MISC_FEATURE (87)..(87): X at position 87 is any amino acid or a deletion
  MISC_FEATURE (91)..(91): X at position 91 is any amino acid or a deletion
  MISC_FEATURE (93)..(96): X at position 93 to 96 is any amino acid or a deletion
  MISC_FEATURE (98)..(98): X at position 98 is any amino acid or a deletion
  MISC_FEATURE (105)..(109): X at position 105 to 109 is any amino acid or a deletion
DIXXTQXXXXXSXSXSXXSXXXSXSSXXXSXXXXXWYQQKPXXXXXXXIYXTSXXXXGVPPXRFXGXGSGTXXXLXISXXXXXDXAXYYCXQXXXXPXTFGGGTXXXXX

SEQ ID NO: 34 - protein, 122 aa, Artificial Sequence
  Consensus alignment of SEQ ID NOS: 5 and 19
  MISC_FEATURE (2)..(2): X at position 2 is any amino acid or a deletion
  MISC_FEATURE (9)..(9): X at position 9 is any amino acid or a deletion
  MISC_FEATURE (11)..(11): X at position 11 is any amino acid or a deletion
  MISC_FEATURE (13)..(13): X at position 13 is any amino acid or a deletion
  MISC_FEATURE (16)..(17): X at position 16 to 17 is any amino acid or a deletion
  MISC_FEATURE (20)..(20): X at position 20 is any amino acid or a deletion
  MISC_FEATURE (28)..(28): X at position 28 is any amino acid or a deletion
  MISC_FEATURE (35)..(35): X at position 35 is any amino acid or a deletion
  MISC_FEATURE (38)..(38): X at position 38 is any amino acid or a deletion
  MISC_FEATURE (43)..(43): X at position 43 is any amino acid or a deletion
  MISC_FEATURE (46)..(46): X at position 46 is any amino acid or a deletion
  MISC_FEATURE (51)..(51): X at position 51 is any amino acid or a deletion
  MISC_FEATURE (55)..(55): X at position 55 is any amino acid or a deletion
  MISC_FEATURE (57)..(57): X at position 7 is any amino acid or a deletion
  MISC_FEATURE (62)..(63): X at position 62 to 63 is any amino acid or a deletion
  MISC_FEATURE (65)..(65): X at position 65 is any amino acid or a deletion
  MISC_FEATURE (72)..(73): X at position 72 to 73 is any amino acid or a deletion
  MISC_FEATURE (84)..(85): X at position 84 to 85 is any amino acid or a deletion
  MISC_FEATURE (88)..(88): X at position 88 is any amino acid or a deletion
  MISC_FEATURE (91)..(91): X at position 91 is any amino acid or a deletion
  MISC_FEATURE (93)..(93): X at position 93 is any amino acid or a deletion
  MISC_FEATURE (95)..(95): X at position 95 is any amino acid or a deletion
  MISC_FEATURE (99)..(110): X at position 99 to 110 is any amino acid or a deletion
QXQLVQSGXEXKXPGXXVKXSCKASGYXFTTYGMXWVXQAPGXGLXWMGWXNTYXGXPTYAXXFXGRFVFSXXTSASTAYLQIXXLKXEDXAXYXCARXXXXXXXXXXXXYWGQGTLVTVSA

SEQ ID NO: 35 - protein, 107 aa, Artificial Sequence
  Consensus alignment of SEQ ID NOS: 12 and 20
  MISC_FEATURE (1)..(1): X at position 1 is any amino acid or a deletion
  MISC_FEATURE (9)..(11): X at position 9 to 11 is any amino acid or a deletion
  MISC_FEATURE (16)..(18): X at position 16 to 18 is any amino acid or a deletion
  MISC_FEATURE (20)..(22): X at position 20 to 22 is any amino acid or a deletion
  MISC_FEATURE (30)..(32): X at position 30 to 32 is any amino acid or a deletion
  MISC_FEATURE (39)..(42): X at position 39 to 42 is any amino acid or a deletion
  MISC_FEATURE (45)..(45): X at position 45 is any amino acid or a deletion
  MISC_FEATURE (49)..(49): X at position 49 is any amino acid or a deletion
  MISC_FEATURE (53)..(53): X at position 53 is any amino acid or a deletion
  MISC_FEATURE (55)..(55): X at position 55 is any amino acid or a deletion
  MISC_FEATURE (58)..(58): X at position 58 is any amino acid or a deletion
  MISC_FEATURE (65)..(65): X at position 65 is any amino acid or a deletion
  MISC_FEATURE (74)..(74): X at position 74 is any amino acid or a deletion
  MISC_FEATURE (78)..(78): X at position 78 is any amino acid or a deletion
  MISC_FEATURE (80)..(80): X at position 80 is any amino acid or a deletion
  MISC_FEATURE (83)..(85): X at position 83 to 85 is any amino acid or a deletion
  MISC_FEATURE (87)..(87): X at position 87 is any amino acid or a deletion
  MISC_FEATURE (89)..(89): X at position 89 is any amino acid or a deletion
  MISC_FEATURE (92)..(92): X at position 92 is any amino acid or a deletion
  MISC_FEATURE (94)..(94): X at position 94 is any amino acid or a deletion
  MISC_FEATURE (100)..(100): X at position 100 is any amino acid or a deletion
  MISC_FEATURE (104)..(104): X at position 104 is any amino acid or a deletion
  MISC_FEATURE (106)..(106): X at position 106 is any amino acid or a deletion
XIVLTQSPXXXSVTPXXXVXXXCRASQSIXXXLHWYQQXXXXSPXLLIXYASXSXSGXPSRFSGXGSGTDFTLXINSXEXEDXXXYXCXQSXSXPLTFGXGTKXEXK

SEQ ID NO: 36 - protein, 480 aa, Staphylococcus aureus glucosaminidase
AYTVTKPQTTQTVSKIAQVKPNNTGIRASVYEKTAKNGAKYADRTFYVTKERAHGNETYVLLNNTSHNIPLGWFNVKDLNVQNLGKEVKTTQKYTVNKSNNGLSMVPWGTKNQVILTGNNIAQGTFNATKQVSVGKDVYLYGTINNRTGWVNAKDLTAPTAVKPTTSAAKDYNYTYVIKNGNGYYYVTPNSDTAKYSLKAFNEQPFAVVKEQVINGQTWYYGKLSNGKLAWIKSTDLAKELIKYNQTGMTLNQVAQIQAGLQYKPQVQRVPGKWTDANFNDVKHAMDTKRLAQDPALKYQFLRLDQPQNISIDKINQFLKGKGVLENQGAAFNKAAQMYGINEVYLISHALLETGNGTSQLAKGADVVNNKVVTNSNTKYHNVFGIAAYDNDPLREGIKYAKQAGWDTVSKAIVGGAKFIGNSYVKAGQNTLYKMRWNPAHPGTHQYATDVDWANINAKIIKGYYDKIGEVGKYFDIPQY